European Patent Specification EP 3 749 786 B1, published January 17, 2024. Title: Turf Health Check. Applicant: Syngenta ZHAW Palmisano, Marilena Wohler, Christian. The sequence listing filed with the application follows.

SEQUENCE LISTING (91 sequences)

SEQ ID NO: 1 - DNA, 912 bp, Sclerotinia homoeocarpa
tagatctacacatggttcttacattatatttaggtcacttgatctacaagtgcggtggaattgacaagcgtactattgaaaagttcgagacggtatgacttctccacctttctcttgctatcttttcccgtccttctcatcgagatcagtgtctgcgatcttggtgctgatggatttatcgggttgcgttttctctcatgcgcggagcatacatccgaattctcaaccctttgaacattaccacattgcctttccagaatccctttgctaacccgttaataggaagccaaggagatgggaaagggttccttcaagtacgcatgggttttggacaagttgaaggctgagcgtgagcgtggtatcaccatcgacattgccctctggaagttcgagacacctaagtacaatgttactgtcattggtatgtgtacgaattctttatgccaactgaagtatattaacccattcgcagatgcccccggtcatcgtgatttcatcaagaacatgatcactggtacctcccaagctgattgtgccattcttatcatcgctgccggtgttggtgagttcgaggctggtatctccaaggatggtcagacccgtgagcacgctcttcttgcgtacactcttggtgttaagcaacttatcgttgccatcaacaagatggacaccaccaagtggtccaaggatcgtttcgaggaaatcatcaaggagacaaccaacttcatcaagaaggttggctacaacgccaagactgttcccttcgtgccgatctctggattcgagggtgataacatgattgagccctcaactaactgcccatggtacaagggctgggagagagagtccaaggagtctggcaaacacaccggcaagacccttcttgaggccatcgacagcatggacctgcct

SEQ ID NO: 2 - DNA, 629 bp, Rhizoctonia solani AG2-2IIIB
tgtagctggctccattagtttggagcatgtgcacaccttttgctctttttttaatccacacacacctgtgaacctgtgaggcagagacatggatgggagaacttttatttactttaaaatgaatgattgggacccctacccccccccccctctgtctactcaactctaatataaacccaatttattttaaaatgaatgtaatggatgtaacgcatctaatactaagtttcaacaacggatctcttggctctcgcatcgatgaagaacgcagcgaaatgcgataagtaatgtgaattgcagaattcagtgaatcatcgaatctttgaacgcaccttgcgctccttggtattccttggagcatgcctgtttgagtatcatgaaatcttcaaagtaaacctttttgttaactcaatttggtttcactttggtattggaggttcttgcagcttcacacgctgctcctctttgttcattagctggatctcagtgttatgcttggttcctctcggcgtgataaattatctatcgctgaggactcccgataaaaaggttggccaaggtaaatgcagatgaaccgcttctaatagtccattgacttggacaataaaataattattattttacgatct

SEQ ID NO: 3 - DNA, 613 bp, Microdochium nivale var. nivale
ggtaaccaaatcggtgctgctttctggtgcgtacacctcgactcgaagacgaccacgaccttcgcgacgaaaatgaactcggcagccaaaaaccgtgccgtcgagaatctttagtcgcagaggaatctaacataagggtggagaccggcaaggctaacactatcttccctgatacaggcagaccatctccggcgagcacggtcttgacagcgatggagtgtaagttcaataaccgactcgcagttccttgcgagagaccgcttccctgacggcttctcgggccagatgaaatgcaacagtactgacattctgccaatagctacaacggcaactctgagctccagctcgagcgcatgagcgtctacttcaacgaggtatgtcaccatgggcgacttcgggcttcacacattcggccagctactaactgaccacccacataacttaggcttccggcaacaagtacgttccccgcgccgtcctcgtcgatctcgagcccggtaccatggatgccgtccgtgctggtcccttcggccagctgttccgtcccgacaacttcgtcttcggtcagtccggtgctggcaacaattgggccaagggtcactacactgagggt

SEQ ID NO: 4 - DNA, 455 bp, Pythium aphanidermatum
cttcagtgaactccatctcgtccataccctcaccagtgtaccagtgcaagaaggccttacgacggaacatggccgtgaactgctcgctgacacgcttgaacatctcctggatggcagtcgagttaccgatgaacgtggcgctcatcttgagaccctttggtgggatgtcacaaacgctggccttgatgttgttcgggatccactcaacgaagtacgacgagttcttgttctgaacgttgagcatctgctcgtcgacctccttggtgctcatacgaccacggaacatacaagcggcggtcaggtaacgaccgtgacgaggatcagcggcacacatcatgttcttggcgtcgaactgctgctgggtcagctctggcaccgtaagggcacggtactgctgcgagccgcgcgaggtgagcggagcgaaaccgaccatgaagaagtggaacgggggaaaa

SEQ ID NO: 5 - DNA, 518 bp, Gaeumannomyces graminis var. avenae
ttagtgacccttggcccagttgttgccagcaccagactggccgaaaacgaagttgtcggggcggaacagctggccgaagggaccggcacgaacggcgtccatggtgccgggctcgagatcgacgaggacggcacgggggacatgcttgttgccggaggcctggagcggaaaggttatgggtcagaatacatgatacgaaggtgggaaataccggctgctaatgccggacagaagcttcaactcagggcctgtctgcatacctcgttgaagtagacgctcatgcgctcgagctggagctccgaggtgccgttgtacctgtatcaatatgtcagagcggtgaacggacggcgggccgagccacaagcaggacgaaatacgtacacgccattgctgtcgagaccgtgctcgctagaaatggtctgcctgtcaaagaagtcagtacgggtcacgggcagtggcagtcgtggtcggcggcggatcgtcgcgcggcgtcgtttcataccagaaagcagcaccgt

SEQ ID NO: 6 - DNA, 550 bp, Microdochium nivale var. majus
ggtaaccaaatcggtgctgctttctggtgcgtacaactccgatactcaacgacggccgcagtgacctttgcgacgaaaacaaactcggcggtcaaacccgtatcgccgaaaatcttcggtcgcagaggaatctggcaaaagggtggaaataaacaagcaaggctaacactctcttccccgacacaggcaaaccatctccagtgagcacggtctcgacagcaatggcgtgtaagttcaataaccgactcgcacttcttgcgaaaggccacttccctgatggcgtatcacgccagatgaaatacacaagtactgacatcctgtcaatagctacaacggcacctccgagctccagctcgagcgcatgagtgtctacttcaatgaggcttccggcaacaagtacgttcctcgtgccgtccttgtcgatctcgagcccggtaccatggatgccgtccgtgctggtcccttcggccagctgttccgccccgacaacttcgtcttcggtcagtccggtgctggcaacaactgggccaagggtcactacactgagggt

SEQ ID NO: 7 - DNA, 485 bp, Magnaporthe poae
ttagtgacccttggcccagttgttgccagcaccggactggccgaaaacgaagttgtcggggcggaacagctggccgaagggaccagcacggacagcatccatggtgccgggctcgagatcgaccaggacggcacgggggacatgcttgttgccggaggcctagagcgcggggaggcaatggtgtcagaaaaacaacacgtggttgcgaaagagagacgcgttcggagtctatctgcatacctcgttgaagtagacgctcatgcgctcgagctggagctccgaggtaccgttgtaactgcaccaatatgtcagagcggtgaacggacatgtggccgaggatctcccaaacagaatacatacactccattgctgtcgagaccgtgctcgctggagatggtttgcctgcccaggaagtcagtatcaatgatggatgatcacggtcgtggtgggtgcgagcggtggttcgtaccagaaagcagcaccgt

SEQ ID NO: 8 - DNA, 539 bp, Gaeumannomyces graminis var. avenae
cctcagtgaactccatctcgtccataccctcgccagtgtaccaatgaaggaaagccttgcgcctgaacatggcagtgaactgctcaccaacacgcttgaagagctcttgtatggcagtcgagtttccgatgaaggtcgacgacatcttcaggccccggggagggattgagcagagggcggtctggatgttgttgggaatccactcgacgaagtacgacgagttcttgttctggatgttgcgcatctggtcctcgacctccttcatggagaccttaccacggctatcgcacacagggatggttagttagtgccttctaggttgggcatattaaatgggccagataaataagcccaatgcctagatgcaagactcacaaaatagcagagcaggtcaggtagcgaccgttgcggaagtccgaggcagccatcatgttcttggggtcgaacatctgctgggtcaactcgggcaccgtgacggcgcggaatgagtgggcgccgcggctagtcaggggagcgaagccgaccatgaagaagtggag

SEQ ID NO: 9 - DNA, 236 bp, Rhizoctonia solani AG2-2IV
gttgtagggctcaacaaccgtgtcggagaccttgggggaaggaacgaccgagaatgtgcacatcatacgatcggggtattcttcacggatcttggagatcaaaagggtgcccataccggcaccggttcctccaccgagcgagtgggtaatctggaagccctgaagacactcgcatccctcggcctctttgcgcgcgacatcgagaactgcgtcaacaagctcggcaccttcggtgt

SEQ ID NO: 10 - DNA, 604 bp, Pythium aphanidermatum
tgctttttcaggtgtagttggtacaactttatctgttttaattagaatggaattagcacaacctggtaatcaaatttttatgggaaatcatcaattatataatgttgttgtaacagcacatgcttttataatgattttcttcatggttatgcctgtattaattggtggttttggtaactggtttattcctttaatgattggtgctccagatatggcttttcctagaatgaataatattagtttttggttattacctccttcattattattattagtatcatctgctatagtagaatcaggtgctggtacaggttggactgtatatccaccattatcaagtgtacaagcacactcaggaccttcagtagatttagctatttttagtttacatttatctggtatttcttcattattaggtgctattaattttttatcaactatttataatatgagagctcctggattaagttttcatagattgccattatttgtttggtctgtttttattacagcttttttattattgttaacattaccagtattagcaggtgctattacaatgttattaacagatagaaatttaaatacttctttttatgatcct

SEQ ID NO: 11 - DNA, 657 bp, Colletotrichum graminicola
aatattctcgacatatgcagcctttccgttgagatactatgtacgatcactgttagcatctcttttcaaaaaaggtcttgttggtgtccacgaacctgaaggtagtacgcgtgctcccacatgtcaataccaaagatgggcacgcccttggtgacagggtcctggtctttcgtcgtgataatgctgaggcccgttatgtcatccttaacaagccacccccagccgctaccggtgatacccagcagcgtggtgttgaaagcctgcttgaactggtcgagcccgccccagacgcgggtgatctcggcgacgagctttggcgccgcatcgggcgaggcatcaccgctcgaggctggggaaaggttctcccagaatagggaatggttgatgtggccgccgccgttgaagtttagggccgcgaggacggcgatgcgattctggagcgggtttgcattgtaagtctcgatggccttgttcagatttgtaacgtatgcttgatggctgtaggtggcttcatgtcaactctcttcttcgctgcttcatatttcatggttatctcactgtttgctgtggtgcagctccatgatctgagctgagatgtgaggctcgagggcctgcaggaggggtcagcgggcgcgatcgcgagcacgagtaagggat

SEQ ID NO: 12 - DNA, 663 bp, Colletotrichum cereale
cgttccagatgttctcgacgtacgccgcttttccattgaggtactgaggccgagcattgttagtaccttccaacaaagcagatccgtcagtgtttacgaacctggaggtagtacgcgtgctcccacatgtccacgccgaagatgggcacgcccttggtgacagggtcctggtctttcgtcgtgatgatgctcagacccgttacgtcgtccttgaccagccatccccagccgctgccggtgatacccagaagcgtggcgttgaaagcctgcttgaactggtcgagcccgccccagacccgggcgatctcagcgacgagcttcggcgcggcgtctggcgaggcgtctgggctcgaggcaggggacaggttttcccagaagagggagtggttgatgtggccgccgccgttgaagttgagggctgggaggacggcgatgcggttctggagggggttcgcgttgtaggtctcgacggccttgtttagatttgtaacgtatgcttcgtgactgcgatggtttgatttcaaccctgttcttctttggtttctagtgcctagctctcttactgtttgctgtggtgcagctccatgatctgggctgagatgtgcggctcgagagcctggaagaggggtcagcgggtgcgaccgcgaacacaagtacggggat

SEQ ID NO: 13 - DNA, 703 bp, Pythium ultimum var. ultimum
tcagaagaaaggtttcctacctcagacagcgtacgccatcctttactttcatttcgcgctggggtttccacaccctaacacttgcacacatgttagactccttggtccgtgtttcaagacgggccgaatcgctccatttcgtcaaagtcccgaacggcaaaagttactctagatctcaatcgaccaatcactccgtcagcatagcaagctatccaaacaggtaaccaaacgagagtcccaaacactttaaagcacattgtaggcacctcagtcccaaccacgacaactaactaccaagatataacagccaagagcaagctcctaacctacctcctcagtagccatttctcacagcatacgaactgactctgacgtcccaccgcaacacagggcaccaacaagcaaacgcagaacagcacaaagagcagaaaaccacttcttacatactgcacgcacctactcgccaatgaaatatgctacagattatagacactggatacgattcgcttccctttcagcagtttcaggtactctttaactctcttttcaaagttcttttcatctttccctcacggtacttgttcgctatcggtctcgcaccaatatttagctttagatggaatttaccacctactttgcgctgcagtcccaaacaacgcgactcaaagaaaacgtgtcgtacgcacaagctactcaggcacaa

SEQ ID NO: 14 - DNA, 18 bp, Artificial Sequence
  Primer for fungal detection
gctcagccttcaacttgt

SEQ ID NO: 15 - DNA, 45 bp, Artificial Sequence
  Primer for fungal detection
gcctttccagaatccctttgctttttgaaggaaccctttcccatc

SEQ ID NO: 16 - DNA, 19 bp, Artificial Sequence
  Primer for fungal detection
ggtggaattgacaagcgta

SEQ ID NO: 17 - DNA, 43 bp, Artificial Sequence
  Primer for fungal detection
atgctccgcgcatgagagttttcttctcatcgagatcagtgtc

SEQ ID NO: 18 - DNA, 21 bp, Artificial Sequence
  Primer for fungal detection
ccgttaataggaagccaagga

SEQ ID NO: 19 - DNA, 19 bp, Artificial Sequence
  Primer for fungal detection
tccatcagcaccaagatcg

SEQ ID NO: 20 - DNA, 20 bp, Artificial Sequence
  Primer for fungal detection
atttaccttggccaaccttt

SEQ ID NO: 21 - DNA, 41 bp, Artificial Sequence
  Primer for fungal detection
gcttcacacgctgctcctttttggagtcctcagcgatagat

SEQ ID NO: 22 - DNA, 19 bp, Artificial Sequence
  Primer for fungal detection
tgtagctggctccattagt

SEQ ID NO: 23 - DNA, 41 bp, Artificial Sequence
  Primer for fungal detection
ggggtaggggtcccaatcatttttgcacaccttttgctctt

SEQ ID NO: 24 - DNA, 22 bp, Artificial Sequence
  Primer for fungal detection
tagctggatctcagtgttatgc

SEQ ID NO: 25 - DNA, 19 bp, Artificial Sequence
  Primer for fungal detection
ctcccatccatgtctctgc

SEQ ID NO: 26 - DNA, 18 bp, Artificial Sequence
  Primer for fungal detection
aatgtgtgaagcccgaag

SEQ ID NO: 27 - DNA, 42 bp, Artificial Sequence
  Primer for fungal detection
gcttccctgacggcttctcttttctcagagttgccgttgtag

SEQ ID NO: 28 - DNA, 22 bp, Artificial Sequence
  Primer for fungal detection
gtcgcagaggaatctaacataa

SEQ ID NO: 29 - DNA, 44 bp, Artificial Sequence
  Primer for fungal detection
aggaactgcgagtcggttattgtttttacaggcagaccatctcc

SEQ ID NO: 30 - DNA, 22 bp, Artificial Sequence
  Primer for fungal detection
acagtactgacattctgccaat

SEQ ID NO: 31 - DNA, 19 bp, Artificial Sequence
  Primer for fungal detection
acactccatcgctgtcaag

SEQ ID NO: 32 - DNA, 20 bp, Artificial Sequence
  Primer for fungal detection
tgaactccatctcgtccata

SEQ ID NO: 33 - DNA, 18 bp, Artificial Sequence
  Primer for fungal detection
tcgtatgagcaccaagga

SEQ ID NO: 34 - DNA, 19 bp, Artificial Sequence
  Primer for fungal detection
gatgttcaagcgtgtcagc

SEQ ID NO: 35 - DNA, 19 bp, Artificial Sequence
  Primer for fungal detection
gctggccttgatgttgttc

SEQ ID NO: 36 - DNA, 42 bp, Artificial Sequence
  Primer for fungal detection
cggtaactcgactgccatccttttccttacgacggaacatgg

SEQ ID NO: 37 - DNA, 44 bp, Artificial Sequence
  Primer for fungal detection
ccctttggtgggatgtcacaattttctcgtcgtacttcgttgag

SEQ ID NO: 38 - DNA, 19 bp, Artificial Sequence
  Primer for fungal detection
ttgaagtagacgctcatgc

SEQ ID NO: 39 - DNA, 19 bp, Artificial Sequence
  Primer for fungal detection
gtgctgctttctggtatga

SEQ ID NO: 40 - DNA, 18 bp, Artificial Sequence
  Primer for fungal detection
cgttcaccgctctgacat

SEQ ID NO: 41 - DNA, 19 bp, Artificial Sequence
  Primer for fungal detection
cgctagaaatggtctgcct

SEQ ID NO: 42 - DNA, 43 bp, Artificial Sequence
  Primer for fungal detection
ttcgtcctgcttgtggctcttttgccgttgtacctgtatcaat

SEQ ID NO: 43 - DNA, 41 bp, Artificial Sequence
  Primer for fungal detection
ttgctgtcgagaccgtgctttttgacccgtactgacttctt

SEQ ID NO: 44 - DNA, 18 bp, Artificial Sequence
  Primer for fungal detection
ggtaaccaaatcggtgct

SEQ ID NO: 45 - DNA, 19 bp, Artificial Sequence
  Primer for fungal detection
gcgagtcggttattgaact

SEQ ID NO: 46 - DNA, 19 bp, Artificial Sequence
  Primer for fungal detection
tttcgtcgcaaaggtcact

SEQ ID NO: 47 - DNA, 21 bp, Artificial Sequence
  Primer for fungal detection
aacaagcaaggctaacactct

SEQ ID NO: 48 - DNA, 41 bp, Artificial Sequence
  Primer for fungal detection
gggtttgaccgccgagttttttgcgtacaactccgatactc

SEQ ID NO: 49 - DNA, 43 bp, Artificial Sequence
  Primer for fungal detection
ggaatctggcaaaagggtggatttttgctcactggagatggtt

SEQ ID NO: 50 - DNA, 19 bp, Artificial Sequence
  Primer for fungal detection
ttgaagtagacgctcatgc

SEQ ID NO: 51 - DNA, 18 bp, Artificial Sequence
  Primer for fungal detection
gctgctttctggtacgaa

SEQ ID NO: 52 - DNA, 20 bp, Artificial Sequence
  Primer for fungal detection
tcaccgctctgacatattgg

SEQ ID NO: 53 - DNA, 18 bp, Artificial Sequence
  Primer for fungal detection
gctggagatggtttgcct

SEQ ID NO: 54 - DNA, 42 bp, Artificial Sequence
  Primer for fungal detection
ggagatcctcggccacatgttttcgaggtaccgttgtaactg

SEQ ID NO: 55 - DNA, 42 bp, Artificial Sequence
  Primer for fungal detection
ttgctgtcgagaccgtgcttttaccgtgatcatccatcattg

SEQ ID NO: 56 - DNA, 19 bp, Artificial Sequence
  Primer for fungal detection
gacgaagtacgacgagttc

SEQ ID NO: 57 - DNA, 19 bp, Artificial Sequence
  Primer for fungal detection
ctccacttcttcatggtcg

SEQ ID NO: 58 - DNA, 19 bp, Artificial Sequence
  Primer for fungal detection
cgatagccgtggtaaggtc

SEQ ID NO: 59 - DNA, 19 bp, Artificial Sequence
  Primer for fungal detection
aggcagccatcatgttctt

SEQ ID NO: 60 - DNA, 44 bp, Artificial Sequence
  Primer for fungal detection
gcccaacctagaaggcactaactttttcctcgacctccttcatg

SEQ ID NO: 61 - DNA, 41 bp, Artificial Sequence
  Primer for fungal detection
ggtcaggtagcgaccgttgttttgagttgacccagcagatg

SEQ ID NO: 62 - DNA, 18 bp, Artificial Sequence
  Primer for fungal detection
ttgtagggctcaacaacc

SEQ ID NO: 63 - DNA, 18 bp, Artificial Sequence
  Primer for fungal detection
gacgcagttctcgatgtc

SEQ ID NO: 64 - DNA, 44 bp, Artificial Sequence
  Primer for fungal detection
ggcacccttttgatctccaagattttggaacgaccgagaatgtg

SEQ ID NO: 65 - DNA, 40 bp, Artificial Sequence
  Primer for fungal detection
ataccggcaccggttcctttttgatgcgagtgtcttcagg

SEQ ID NO: 66 - DNA, 20 bp, Artificial Sequence
  Primer for fungal detection
ccgtgaagaataccccgatc

SEQ ID NO: 67 - DNA, 18 bp, Artificial Sequence
  Primer for fungal detection
ccgagcgagtgggtaatc

SEQ ID NO: 68 - DNA, 22 bp, Artificial Sequence
  Primer for fungal detection
aattagcacaacctggtaatca

SEQ ID NO: 69 - DNA, 22 bp, Artificial Sequence
  Primer for fungal detection
acttaatccaggagctctcata

SEQ ID NO: 70 - DNA, 48 bp, Artificial Sequence
  Primer for fungal detection
gccatatctggagcaccaatcattttaatgttgttgtaacagcacatg

SEQ ID NO: 71 - DNA, 47 bp, Artificial Sequence
  Primer for fungal detection
aatcaggtgctggtacaggttgttttaatctactgaaggtcctgagt

SEQ ID NO: 72 - DNA, 22 bp, Artificial Sequence
  Primer for fungal detection
aaccaccaattaatacaggcat

SEQ ID NO: 73 - DNA, 22 bp, Artificial Sequence
  Primer for fungal detection
accattatcaagtgtacaagca

SEQ ID NO: 74 - DNA, 21 bp, Artificial Sequence
  Primer for fungal detection
tgtacgatcactgttagcatc

SEQ ID NO: 75 - DNA, 18 bp, Artificial Sequence
  Primer for fungal detection
ctcgaccagttcaagcag

SEQ ID NO: 76 - DNA, 41 bp, Artificial Sequence
  Primer for fungal detection
ggcgtgcccatctttggtattttgtgtccacgaacctgaag

SEQ ID NO: 77 - DNA, 43 bp, Artificial Sequence
  Primer for fungal detection
ggtgacagggtcctggtctttttgtggcttgttaaggatgaca

SEQ ID NO: 78 - DNA, 18 bp, Artificial Sequence
  Primer for fungal detection
ttgacatgtgggagcacg

SEQ ID NO: 79 - DNA, 20 bp, Artificial Sequence
  Primer for fungal detection
tcgtcgtgataatgctgagg

SEQ ID NO: 80 - DNA, 19 bp, Artificial Sequence
  Primer for fungal detection
cgttccagatgttctcgac

SEQ ID NO: 81 - DNA, 18 bp, Artificial Sequence
  Primer for fungal detection
gtcaaggacgacgtaacg

SEQ ID NO: 82 - DNA, 47 bp, Artificial Sequence
  Primer for fungal detection
gcgtactacctccaggttcgtattttgagcattgttagtaccttcca

SEQ ID NO: 83 - DNA, 41 bp, Artificial Sequence
  Primer for fungal detection
atgtccacgccgaagatggttttctgagcatcatcacgacg

SEQ ID NO: 84 - DNA, 19 bp, Artificial Sequence
  Primer for fungal detection
aacactgacggatctgctt

SEQ ID NO: 85 - DNA, 18 bp, Artificial Sequence
  Primer for fungal detection
tgacagggtcctggtctt

SEQ ID NO: 86 - DNA, 18 bp, Artificial Sequence
  Primer for fungal detection
caaacgagagtcccaaac

SEQ ID NO: 87 - DNA, 22 bp, Artificial Sequence
  Primer for fungal detection
atccagtgtctataatctgtag

SEQ ID NO: 88 - DNA, 44 bp, Artificial Sequence
  Primer for fungal detection
gagtcagttcgtatgctgtgagtttttaacagccaagagcaagc

SEQ ID NO: 89 - DNA, 44 bp, Artificial Sequence
  Primer for fungal detection
cgcaacacagggcaccaacttttgtgcagtatgtaagaagtggt

SEQ ID NO: 90 - DNA, 19 bp, Artificial Sequence
  Primer for fungal detection
ggctactgaggaggtaggt

SEQ ID NO: 91 - DNA, 20 bp, Artificial Sequence
  Primer for fungal detection
agaacagcacaaagagcaga